European Patent Application EP 4 269 623 A2, published November 1, 2023. Title: ANALYSIS OF A BIOLOGICAL SAMPLE OF AN ORGANISM FOR CHROMOSOMAL DELETIONS OR AMPLIFICATIONS ASSOCIATED WITH CANCER. Applicant: The Chinese University Of Hong Kong. Application EP, filed November 30, 2011. The sequence listing filed with the application follows.

SEQUENCE LISTING (4 sequences)

SEQ ID NO: 1 - DNA, 11 bp, synthetic construct
  misc_feature 1..11: note = synthetic normal cell, cancer cell, region with loss of heterozygosity (LOH) in cancer and cancer cell with LOH haplotype I (Hap I)
  source 1..11: mol_type = other DNA
atgcctgaatc

SEQ ID NO: 2 - DNA, 11 bp, synthetic construct
  misc_feature 1..11: note = synthetic normal cell and cancer cell haplotype II (Hap II)
  source 1..11: mol_type = other DNA
tacgtcatgct

SEQ ID NO: 3 - DNA, 14 bp, synthetic construct
  misc_feature 1..14: note = synthetic non-tumour tissue and cancer cell haplotype I (Hap I)
  source 1..14: mol_type = other DNA
atgcgtcatgagta

SEQ ID NO: 4 - DNA, 14 bp, synthetic construct
  misc_feature 1..14: note = synthetic non-tumour tissue haplotype II (Hap II)
  source 1..14: mol_type = other DNA
tacttgataagcat